European Patent Application EP 4 321 620 A1, published February 14, 2024. Title: METHOD FOR PRODUCING TAGATOSE BY IMMOBILIZING MULTIPLE ENZYMES BY USING ARTIFICIAL OIL BODY. Applicant: TIANJIN INSTITUTE OF INDUSTRIAL BIOTECHNOLOGY, CHINESE ACADEMY OF SCIENCES. The sequence listing filed with the application follows.

SEQUENCE LISTING (1 sequence)

SEQ ID NO: 1 - DNA, 450 bp, Artificial Sequence
  synthetic
gcaatggcagatattggtagcgaatttcacatgtggatctataatagcgttccgacctgcaaaccgaattggattaagagcaatcagcataatccgacccgtgccccgaatccgagtagcaccattcagagctgtctggccggtattggccatctgcagattcgcccgaaacagacctgtccgcagcgcagtccgagtgcactgcatgccacctttgcctgttatagcctgcagcatgttaccccgccgccgccgcatccgacccctcctcctcctccaccgccgttacagcagcagacccgcgcccctcatctgcagctgcagccgcgtgcacagcgcgttgttaaagccgccaccgccgttaccgccggtggcagcttactggtgctgagcggtctgaccctggcaggtaccgtgattgcactgaccattgcaaccccgctgctggtt